European Patent Specification EP 3 464 360 B1, published November 12, 2025. Title: ANTI-TIM-3 ANTIBODIES AND METHODS OF USE THEREOF. Applicant: Agenus Inc. The sequence listing filed with the application follows.

SEQUENCE LISTING (102 sequences)

SEQ ID NO: 1 - protein, 6 aa, Artificial Sequence
  BADD456-2919 CDRH1
SSYAMS

SEQ ID NO: 2 - protein, 13 aa, Artificial Sequence
  BADD456-2919 CDRH2
WVSAISGSGGSTY

SEQ ID NO: 3 - protein, 12 aa, Artificial Sequence
  BADD456-2919 CDRH3
AKGGDYGGNYFD

SEQ ID NO: 4 - protein, 6 aa, Artificial Sequence
  AM-1 CDRH1
KAGQSS

SEQ ID NO: 5 - protein, 6 aa, Artificial Sequence
  AM-2 CDRH1
RQNAWS

SEQ ID NO: 6 - protein, 6 aa, Artificial Sequence
  AM-3 CDRH1
MSGQTS

SEQ ID NO: 7 - protein, 6 aa, Artificial Sequence
  AM-4 CDRH1
GAGQSS

SEQ ID NO: 8 - protein, 6 aa, Artificial Sequence
  AM-5 CDRH1
SAQQAS

SEQ ID NO: 9 - protein, 6 aa, Artificial Sequence
  AM-6 CDRH1
ARNAWS

SEQ ID NO: 10 - protein, 6 aa, Artificial Sequence
  AM-7 CDRH1
RSQQAS

SEQ ID NO: 11 - protein, 6 aa, Artificial Sequence
  AM-8 CDRH1
TTQQAS

SEQ ID NO: 12 - protein, 6 aa, Artificial Sequence
  AM-9 CDRH1
GGQQAS

SEQ ID NO: 13 - protein, 12 aa, Artificial Sequence
  BADD197-1181 CDRL1
RASQSVSSSYLA

SEQ ID NO: 14 - protein, 11 aa, Artificial Sequence
  BADD412-2513 CDRL1
RASQSVSSYLA

SEQ ID NO: 15 - protein, 11 aa, Artificial Sequence
  BADD456-2928 CDRL1
RASQGISNYLA

SEQ ID NO: 16 - protein, 12 aa, Artificial Sequence
  BADD466-3169 CDRL1
GASQSVSSSYLA

SEQ ID NO: 17 - protein, 7 aa, Artificial Sequence
  BADD197-1181 CDRL2
GASSRAT

SEQ ID NO: 18 - protein, 7 aa, Artificial Sequence
  BADD456-2928 CDRL2
AASTLQS

SEQ ID NO: 19 - protein, 7 aa, Artificial Sequence
  BADD466-3165 CDRL2
GASTRAT

SEQ ID NO: 20 - protein, 7 aa, Artificial Sequence
  BADD466-3166 CDRL2
DASSRAT

SEQ ID NO: 21 - protein, 7 aa, Artificial Sequence
  BADD466-3167 CDRL2
DASNRAT

SEQ ID NO: 22 - protein, 9 aa, Artificial Sequence
  BADD197-1181 CDRL3
QQYGSSPLT

SEQ ID NO: 23 - protein, 9 aa, Artificial Sequence
  BADD392-2234 CDRL3
QQYGSSPIT

SEQ ID NO: 24 - protein, 120 aa, Artificial Sequence
  BADD456-2919 VH
EVQLVESGGGLVQPGGSLRLSCAASGFTFSSYAMSWVRQAPGKGLEWVSAISGSGGSTYYADSVKGRFTISRDNSKNTLYLQMNSLRAEDTAVYYCAKGGDYGGNYFDYWGQGTLVTVSS

SEQ ID NO: 25 - protein, 120 aa, Artificial Sequence
  BADD466-3162 VH
EVQLVESGGGLVQPGGSLRLSCAASGFTFSSYAMSWVRRAPGKGLEWVSAISGSGGSTYYADSVKGRFTISRDNSKNTLYLQMNSLRAEDTAVYYCAKGGDYGGNYFDYWGQGTLVTVSS

SEQ ID NO: 26 - protein, 120 aa, Artificial Sequence
  BADD466-3163 VH
EVQLVESGGGLVQPRGSLRLSCAASGFTFSSYAMSWVRQAPGKGLEWVSAISGSGGSTYYADSVKGRFTISRDNSKNTLYLQMNSLRAEDTAVYYCAKGGDYGGNYFDYWGQGTLVTVSS

SEQ ID NO: 27 - protein, 120 aa, Artificial Sequence
  AM-1-VH
EVQLVESGGGLVQPGGSLRLSCAASGFTFKAGQSSWVRRAPGKGLEWVSAISGSGGSTYYADSVKGRFTISRDNSKNTLYLQMNSLRAEDTAVYYCAKGGDYGGNYFDYWGQGTLVTVSS

SEQ ID NO: 28 - protein, 120 aa, Artificial Sequence
  AM-2-VH
EVQLVESGGGLVQPGGSLRLSCAASGFTFRQNAWSWVRRAPGKGLEWVSAISGSGGSTYYADSVKGRFTISRDNSKNTLYLQMNSLRAEDTAVYYCAKGGDYGGNYFDYWGQGTLVTVSS

SEQ ID NO: 29 - protein, 120 aa, Artificial Sequence
  AM-3-VH
EVQLVESGGGLVQPGGSLRLSCAASGFTFMSGQTSWVRRAPGKGLEWVSAISGSGGSTYYADSVKGRFTISRDNSKNTLYLQMNSLRAEDTAVYYCAKGGDYGGNYFDYWGQGTLVTVSS

SEQ ID NO: 30 - protein, 120 aa, Artificial Sequence
  AM-4-VH
EVQLVESGGGLVQPGGSLRLSCAASGFTFGAGQSSWVRRAPGKGLEWVSAISGSGGSTYYADSVKGRFTISRDNSKNTLYLQMNSLRAEDTAVYYCAKGGDYGGNYFDYWGQGTLVTVSS

SEQ ID NO: 31 - protein, 120 aa, Artificial Sequence
  AM-5-VH
EVQLVESGGGLVQPGGSLRLSCAASGFTFSAQQASWVRRAPGKGLEWVSAISGSGGSTYYADSVKGRFTISRDNSKNTLYLQMNSLRAEDTAVYYCAKGGDYGGNYFDYWGQGTLVTVSS

SEQ ID NO: 32 - protein, 120 aa, Artificial Sequence
  AM-6-VH
EVQLVESGGGLVQPGGSLRLSCAASGFTFARNAWSWVRRAPGKGLEWVSAISGSGGSTYYADSVKGRFTISRDNSKNTLYLQMNSLRAEDTAVYYCAKGGDYGGNYFDYWGQGTLVTVSS

SEQ ID NO: 33 - protein, 120 aa, Artificial Sequence
  AM-7-VH
EVQLVESGGGLVQPGGSLRLSCAASGFTFRSQQASWVRRAPGKGLEWVSAISGSGGSTYYADSVKGRFTISRDNSKNTLYLQMNSLRAEDTAVYYCAKGGDYGGNYFDYWGQGTLVTVSS

SEQ ID NO: 34 - protein, 120 aa, Artificial Sequence
  AM-8-VH
EVQLVESGGGLVQPGGSLRLSCAASGFTFTTQQASWVRRAPGKGLEWVSAISGSGGSTYYADSVKGRFTISRDNSKNTLYLQMNSLRAEDTAVYYCAKGGDYGGNYFDYWGQGTLVTVSS

SEQ ID NO: 35 - protein, 120 aa, Artificial Sequence
  AM-9-VH
EVQLVESGGGLVQPGGSLRLSCAASGFTFGGQQASWVRRAPGKGLEWVSAISGSGGSTYYADSVKGRFTISRDNSKNTLYLQMNSLRAEDTAVYYCAKGGDYGGNYFDYWGQGTLVTVSS

SEQ ID NO: 36 - protein, 108 aa, Artificial Sequence
  BADD197-1181 VL
EIVLTQSPGTLSLSPGERATLSCRASQSVSSSYLAWYQQKPGQAPRLLIYGASSRATGIPDRFSGSGSGTDFTLTISRLEPEDFAVYYCQQYGSSPLTFGGGTKVEIK

SEQ ID NO: 37 - protein, 107 aa, Artificial Sequence
  BADD412-2513 VL
EIVLTQSPGTLSLSPGERATLSCRASQSVSSYLAWYQQKPGQAPRLLIYGASSRATGIPDRFSGSGSGTDFTLTISRLEPEDFAVYYCQQYGSSPLTFGGGTKVEIK

SEQ ID NO: 38 - protein, 107 aa, Artificial Sequence
  BADD456-2928 VL
DIQMTQSPSSLSASVGDRVTITCRASQGISNYLAWYQQKPGKVPKLLIYAASTLQSGVPSRFSGSGSGTDFTLTISRLEPEDFAVYYCQQYGSSPLTFGGGTKVEIK

SEQ ID NO: 39 - protein, 107 aa, Artificial Sequence
  BADD466-3164 VL
EIVLTQSPATLSLSPGERATLSCRASQSVSSYLAWYQQKPGQAPRLLIYGASSRATGIPDRFSGSGSGTDFTLTISRLEPEDFAVYYCQQYGSSPLTFGGGTKVKIK

SEQ ID NO: 40 - protein, 107 aa, Artificial Sequence
  BADD466-3165 VL
EIVLTQSPATLSLSPGERATLSCRASQSVSSYLAWYQQKPGQAPRLLIYGASTRATGIPARFSGSGSGTDFTLTISRLEPEDFAVYYCQQYGSSPLTFGGGTKVEIK

SEQ ID NO: 41 - protein, 107 aa, Artificial Sequence
  BADD466-3166 VL
EIVLTQSPGTLSLSPGERATLSCRASQSVSSYLAWYQQKPGQAPRLLIYDASSRATGIPDRFSGSGSGTDFTLTISRLEPEDFAVYYCQQYGSSPLTFGGGTKVEIK

SEQ ID NO: 42 - protein, 107 aa, Artificial Sequence
  BADD466-3167 VL
EIVLTQSPATLSLSPGERATLSCRASQSVSSYLAWYQQKPGQAPRLLIYDASNRATGIPARFSGSGSGTDFTLTISRLEPEDFAVYYCQQYGSSPLTFGGGTKVEIK

SEQ ID NO: 43 - protein, 107 aa, Artificial Sequence
  BADD466-3168 VL
EIVLTQSPGTLSLSPGERATLSCRASQSVSSYLAWYQQKPGQAPRLLIYDASNRATGIPARFSGSGSGTDFTLTISRLEPEDFAVYYCQQYGSSPLTFGGGTKVEIK

SEQ ID NO: 44 - protein, 108 aa, Artificial Sequence
  BADD466-3169 VL
EIVLTQSPATLSLSPGERATLSCGASQSVSSSYLAWYQQKPGLAPRLLIYDASSRATGIPDRFSGSGSGTDFTLTISRLEPEDFAVYYCQQYGSSPLTFGGGTKVEIK

SEQ ID NO: 45 - protein, 107 aa, Artificial Sequence
  BADD466-3170 VL
EIVLTQSPATLSLSPGERATLSCRASQSVSSYLAWYQQKPGQAPRLLIYDASNRATGIPARFSGSGSGTDFTLTISSLEPEDFAVYYCQQYGSSPLTFGGGTKVEIK

SEQ ID NO: 46 - protein, 107 aa, Artificial Sequence
  BADD466-3171 VL
EIVLTQSPATLSLSPGERATLSCRASQSVSSYLAWYQQKPGQAPRLLIYDASNRATGIPASFSGSGSGTDFTLTISRLEPEDFAVYYCQQYGSSPLTFGGGTKVEIK

SEQ ID NO: 47 - protein, 107 aa, Artificial Sequence
  BADD466-3172 VL
EIVLTQSPGTLSLSPGERATLSCRASQSVSSYLAWYQQKPGQAPRLLIYGASSRATGIPARFSGSGSGTDFTLTISRLEPEDFAVYYCQQYGSSPITFGGGTKVEIK

SEQ ID NO: 48 - protein, 6 aa, Artificial Sequence
  CDRH1 consensus sequence 1
  VARIANT (1)..(1): Arg, Ser, Ala, Gly, Lys, Met, or Thr
  VARIANT (2)..(2): Gln, Ser, Ala, Gly, Arg, or Thr
  VARIANT (3)..(3): Asn, Tyr, Gly, or Gln
  VARIANT (4)..(4): Ala or Gln
  VARIANT (5)..(5): Trp, Met, Ala, Ser, or Thr
XXXXXS

SEQ ID NO: 49 - protein, 6 aa, Artificial Sequence
  CDRH1 consensus sequence 2
  VARIANT (1)..(1): Arg or Ala
  VARIANT (2)..(2): Gln or Arg
XXNAWS

SEQ ID NO: 50 - protein, 6 aa, Artificial Sequence
  CDRH1 consensus sequence 3
  VARIANT (1)..(1): Lys, Met, or Gly
  VARIANT (2)..(2): Ala or Ser
  VARIANT (5)..(5): Ser or Thr
XXGQXS

SEQ ID NO: 51 - protein, 6 aa, Artificial Sequence
  CDRH1 consensus sequence 4
  VARIANT (1)..(1): Ser, Arg, Thr, or Gly
  VARIANT (2)..(2): Ala, Ser, Thr, or Gly
XXQQAS

SEQ ID NO: 52 - protein, 12 aa, Artificial Sequence
  XASQSVXSSYLA
  VARIANT (1)..(1): Arg or Gly
  VARIANT (7)..(7): absent or Ser
XASQSVXSSYLA

SEQ ID NO: 53 - protein, 7 aa, Artificial Sequence
  CDRL2 consensus sequence
  VARIANT (1)..(1): Asp or Gly
  VARIANT (4)..(4): Asn, Ser, or Thr
XASXRAT

SEQ ID NO: 54 - protein, 9 aa, Artificial Sequence
  CDRL3 consensus sequence
  VARIANT (8)..(8): Leu or Ile
QQYGSSPXT

SEQ ID NO: 55 - protein, 120 aa, Artificial Sequence
  VH consensus sequence
  VARIANT (15)..(15): Gly or Arg
  VARIANT (30)..(30): Arg, Ser, Ala, Gly, Lys, Met, or Thr
  VARIANT (31)..(31): Gln, Ser, Ala, Gly, Arg, or Thr
  VARIANT (32)..(32): Asn, Tyr, Gly, or Gln
  VARIANT (33)..(33): Ala or Gln
  VARIANT (34)..(34): Trp, Met, Ala, Ser, or Thr
  VARIANT (39)..(39): Arg or Gln
EVQLVESGGGLVQPXGSLRLSCAASGFTFXXXXXSWVRXAPGKGLEWVSAISGSGGSTYYADSVKGRFTISRDNSKNTLYLQMNSLRAEDTAVYYCAKGGDYGGNYFDYWGQGTLVTVSS

SEQ ID NO: 56 - protein, 108 aa, Artificial Sequence
  VL consensus sequence
  VARIANT (9)..(9): Ala or Gly
  VARIANT (24)..(24): Arg or Gly
  VARIANT (30)..(30): absent or Ser
  VARIANT (43)..(43): Gln or Leu
  VARIANT (51)..(51): Asp or Gly
  VARIANT (54)..(54): Asn, Ser, or Thr
  VARIANT (61)..(61): Ala or Asp
  VARIANT (62)..(62): Ser or Arg
  VARIANT (78)..(78): Arg or Ser
  VARIANT (97)..(97): Leu or Ile
  VARIANT (106)..(106): Glu or Lys
EIVLTQSPXTLSLSPGERATLSCXASQSVXSSYLAWYQQKPGXAPRLLIYXASXRATGIPXXFSGSGSGTDFTLTISXLEPEDFAVYYCQQYGSSPXTFGGGTKVXIK

SEQ ID NO: 57 - protein, 449 aa, Artificial Sequence
  pab2188 full length IgG1 heavy chain
EVQLVESGGGLVQPGGSLRLSCAASGFTFSSYAMSWVRRAPGKGLEWVSAISGSGGSTYYADSVKGRFTISRDNSKNTLYLQMNSLRAEDTAVYYCAKGGDYGGNYFDYWGQGTLVTVSSASTKGPSVFPLAPSSKSTSGGTAALGCLVKDYFPEPVTVSWNSGALTSGVHTFPAVLQSSGLYSLSSVVTVPSSSLGTQTYICNVNHKPSNTKVDKRVEPKSCDKTHTCPPCPAPELLGGPSVFLFPPKPKDTLMISRTPEVTCVVVDVSHEDPEVKFNWYVDGVEVHNAKTKPREEQYNSTYRVVSVLTVLHQDWLNGKEYKCKVSNKALPAPIEKTISKAKGQPREPQVYTLPPSREEMTKNQVSLTCLVKGFYPSDIAVEWESNGQPENNYKTTPPVLDSDGSFFLYSKLTVDKSRWQQGNVFSCSVMHEALHNHYTQKSLSLSPG

SEQ ID NO: 58 - protein, 449 aa, Artificial Sequence
  pab2188 full length IgG1 N297A heavy chain
EVQLVESGGGLVQPGGSLRLSCAASGFTFSSYAMSWVRRAPGKGLEWVSAISGSGGSTYYADSVKGRFTISRDNSKNTLYLQMNSLRAEDTAVYYCAKGGDYGGNYFDYWGQGTLVTVSSASTKGPSVFPLAPSSKSTSGGTAALGCLVKDYFPEPVTVSWNSGALTSGVHTFPAVLQSSGLYSLSSVVTVPSSSLGTQTYICNVNHKPSNTKVDKRVEPKSCDKTHTCPPCPAPELLGGPSVFLFPPKPKDTLMISRTPEVTCVVVDVSHEDPEVKFNWYVDGVEVHNAKTKPREEQYASTYRVVSVLTVLHQDWLNGKEYKCKVSNKALPAPIEKTISKAKGQPREPQVYTLPPSREEMTKNQVSLTCLVKGFYPSDIAVEWESNGQPENNYKTTPPVLDSDGSFFLYSKLTVDKSRWQQGNVFSCSVMHEALHNHYTQKSLSLSPG

SEQ ID NO: 59 - protein, 446 aa, Artificial Sequence
  pab2188 full length IgG4 S228P heavy chain
EVQLVESGGGLVQPGGSLRLSCAASGFTFSSYAMSWVRRAPGKGLEWVSAISGSGGSTYYADSVKGRFTISRDNSKNTLYLQMNSLRAEDTAVYYCAKGGDYGGNYFDYWGQGTLVTVSSASTKGPSVFPLAPCSRSTSESTAALGCLVKDYFPEPVTVSWNSGALTSGVHTFPAVLQSSGLYSLSSVVTVPSSSLGTKTYTCNVDHKPSNTKVDKRVESKYGPPCPPCPAPEFLGGPSVFLFPPKPKDTLMISRTPEVTCVVVDVSQEDPEVQFNWYVDGVEVHNAKTKPREEQFNSTYRVVSVLTVLHQDWLNGKEYKCKVSNKGLPSSIEKTISKAKGQPREPQVYTLPPSQEEMTKNQVSLTCLVKGFYPSDIAVEWESNGQPENNYKTTPPVLDSDGSFFLYSRLTVDKSRWQEGNVFSCSVMHEALHNHYTQKSLSLSLG

SEQ ID NO: 60 - protein, 449 aa, Artificial Sequence
  AM-1 full length IgG1 N297A heavy chain
EVQLVESGGGLVQPGGSLRLSCAASGFTFKAGQSSWVRRAPGKGLEWVSAISGSGGSTYYADSVKGRFTISRDNSKNTLYLQMNSLRAEDTAVYYCAKGGDYGGNYFDYWGQGTLVTVSSASTKGPSVFPLAPSSKSTSGGTAALGCLVKDYFPEPVTVSWNSGALTSGVHTFPAVLQSSGLYSLSSVVTVPSSSLGTQTYICNVNHKPSNTKVDKRVEPKSCDKTHTCPPCPAPELLGGPSVFLFPPKPKDTLMISRTPEVTCVVVDVSHEDPEVKFNWYVDGVEVHNAKTKPREEQYASTYRVVSVLTVLHQDWLNGKEYKCKVSNKALPAPIEKTISKAKGQPREPQVYTLPPSREEMTKNQVSLTCLVKGFYPSDIAVEWESNGQPENNYKTTPPVLDSDGSFFLYSKLTVDKSRWQQGNVFSCSVMHEALHNHYTQKSLSLSPG

SEQ ID NO: 61 - protein, 449 aa, Artificial Sequence
  AM-2 full length IgG1 N297A heavy chain
EVQLVESGGGLVQPGGSLRLSCAASGFTFRQNAWSWVRRAPGKGLEWVSAISGSGGSTYYADSVKGRFTISRDNSKNTLYLQMNSLRAEDTAVYYCAKGGDYGGNYFDYWGQGTLVTVSSASTKGPSVFPLAPSSKSTSGGTAALGCLVKDYFPEPVTVSWNSGALTSGVHTFPAVLQSSGLYSLSSVVTVPSSSLGTQTYICNVNHKPSNTKVDKRVEPKSCDKTHTCPPCPAPELLGGPSVFLFPPKPKDTLMISRTPEVTCVVVDVSHEDPEVKFNWYVDGVEVHNAKTKPREEQYASTYRVVSVLTVLHQDWLNGKEYKCKVSNKALPAPIEKTISKAKGQPREPQVYTLPPSREEMTKNQVSLTCLVKGFYPSDIAVEWESNGQPENNYKTTPPVLDSDGSFFLYSKLTVDKSRWQQGNVFSCSVMHEALHNHYTQKSLSLSPG

SEQ ID NO: 62 - protein, 449 aa, Artificial Sequence
  AM-3 full length IgG1 N297A heavy chain
EVQLVESGGGLVQPGGSLRLSCAASGFTFMSGQTSWVRRAPGKGLEWVSAISGSGGSTYYADSVKGRFTISRDNSKNTLYLQMNSLRAEDTAVYYCAKGGDYGGNYFDYWGQGTLVTVSSASTKGPSVFPLAPSSKSTSGGTAALGCLVKDYFPEPVTVSWNSGALTSGVHTFPAVLQSSGLYSLSSVVTVPSSSLGTQTYICNVNHKPSNTKVDKRVEPKSCDKTHTCPPCPAPELLGGPSVFLFPPKPKDTLMISRTPEVTCVVVDVSHEDPEVKFNWYVDGVEVHNAKTKPREEQYASTYRVVSVLTVLHQDWLNGKEYKCKVSNKALPAPIEKTISKAKGQPREPQVYTLPPSREEMTKNQVSLTCLVKGFYPSDIAVEWESNGQPENNYKTTPPVLDSDGSFFLYSKLTVDKSRWQQGNVFSCSVMHEALHNHYTQKSLSLSPG

SEQ ID NO: 63 - protein, 449 aa, Artificial Sequence
  AM-4 full length IgG1 N297A heavy chain
EVQLVESGGGLVQPGGSLRLSCAASGFTFGAGQSSWVRRAPGKGLEWVSAISGSGGSTYYADSVKGRFTISRDNSKNTLYLQMNSLRAEDTAVYYCAKGGDYGGNYFDYWGQGTLVTVSSASTKGPSVFPLAPSSKSTSGGTAALGCLVKDYFPEPVTVSWNSGALTSGVHTFPAVLQSSGLYSLSSVVTVPSSSLGTQTYICNVNHKPSNTKVDKRVEPKSCDKTHTCPPCPAPELLGGPSVFLFPPKPKDTLMISRTPEVTCVVVDVSHEDPEVKFNWYVDGVEVHNAKTKPREEQYASTYRVVSVLTVLHQDWLNGKEYKCKVSNKALPAPIEKTISKAKGQPREPQVYTLPPSREEMTKNQVSLTCLVKGFYPSDIAVEWESNGQPENNYKTTPPVLDSDGSFFLYSKLTVDKSRWQQGNVFSCSVMHEALHNHYTQKSLSLSPG

SEQ ID NO: 64 - protein, 449 aa, Artificial Sequence
  AM-5 full length IgG1 N297A heavy chain
EVQLVESGGGLVQPGGSLRLSCAASGFTFSAQQASWVRRAPGKGLEWVSAISGSGGSTYYADSVKGRFTISRDNSKNTLYLQMNSLRAEDTAVYYCAKGGDYGGNYFDYWGQGTLVTVSSASTKGPSVFPLAPSSKSTSGGTAALGCLVKDYFPEPVTVSWNSGALTSGVHTFPAVLQSSGLYSLSSVVTVPSSSLGTQTYICNVNHKPSNTKVDKRVEPKSCDKTHTCPPCPAPELLGGPSVFLFPPKPKDTLMISRTPEVTCVVVDVSHEDPEVKFNWYVDGVEVHNAKTKPREEQYASTYRVVSVLTVLHQDWLNGKEYKCKVSNKALPAPIEKTISKAKGQPREPQVYTLPPSREEMTKNQVSLTCLVKGFYPSDIAVEWESNGQPENNYKTTPPVLDSDGSFFLYSKLTVDKSRWQQGNVFSCSVMHEALHNHYTQKSLSLSPG

SEQ ID NO: 65 - protein, 449 aa, Artificial Sequence
  AM-6 full length IgG1 N297A heavy chain
EVQLVESGGGLVQPGGSLRLSCAASGFTFARNAWSWVRRAPGKGLEWVSAISGSGGSTYYADSVKGRFTISRDNSKNTLYLQMNSLRAEDTAVYYCAKGGDYGGNYFDYWGQGTLVTVSSASTKGPSVFPLAPSSKSTSGGTAALGCLVKDYFPEPVTVSWNSGALTSGVHTFPAVLQSSGLYSLSSVVTVPSSSLGTQTYICNVNHKPSNTKVDKRVEPKSCDKTHTCPPCPAPELLGGPSVFLFPPKPKDTLMISRTPEVTCVVVDVSHEDPEVKFNWYVDGVEVHNAKTKPREEQYASTYRVVSVLTVLHQDWLNGKEYKCKVSNKALPAPIEKTISKAKGQPREPQVYTLPPSREEMTKNQVSLTCLVKGFYPSDIAVEWESNGQPENNYKTTPPVLDSDGSFFLYSKLTVDKSRWQQGNVFSCSVMHEALHNHYTQKSLSLSPG

SEQ ID NO: 66 - protein, 449 aa, Artificial Sequence
  AM-7 full length IgG1 N297A heavy chain
EVQLVESGGGLVQPGGSLRLSCAASGFTFRSQQASWVRRAPGKGLEWVSAISGSGGSTYYADSVKGRFTISRDNSKNTLYLQMNSLRAEDTAVYYCAKGGDYGGNYFDYWGQGTLVTVSSASTKGPSVFPLAPSSKSTSGGTAALGCLVKDYFPEPVTVSWNSGALTSGVHTFPAVLQSSGLYSLSSVVTVPSSSLGTQTYICNVNHKPSNTKVDKRVEPKSCDKTHTCPPCPAPELLGGPSVFLFPPKPKDTLMISRTPEVTCVVVDVSHEDPEVKFNWYVDGVEVHNAKTKPREEQYASTYRVVSVLTVLHQDWLNGKEYKCKVSNKALPAPIEKTISKAKGQPREPQVYTLPPSREEMTKNQVSLTCLVKGFYPSDIAVEWESNGQPENNYKTTPPVLDSDGSFFLYSKLTVDKSRWQQGNVFSCSVMHEALHNHYTQKSLSLSPG

SEQ ID NO: 67 - protein, 449 aa, Artificial Sequence
  AM-8 full length IgG1 N297A heavy chain
EVQLVESGGGLVQPGGSLRLSCAASGFTFTTQQASWVRRAPGKGLEWVSAISGSGGSTYYADSVKGRFTISRDNSKNTLYLQMNSLRAEDTAVYYCAKGGDYGGNYFDYWGQGTLVTVSSASTKGPSVFPLAPSSKSTSGGTAALGCLVKDYFPEPVTVSWNSGALTSGVHTFPAVLQSSGLYSLSSVVTVPSSSLGTQTYICNVNHKPSNTKVDKRVEPKSCDKTHTCPPCPAPELLGGPSVFLFPPKPKDTLMISRTPEVTCVVVDVSHEDPEVKFNWYVDGVEVHNAKTKPREEQYASTYRVVSVLTVLHQDWLNGKEYKCKVSNKALPAPIEKTISKAKGQPREPQVYTLPPSREEMTKNQVSLTCLVKGFYPSDIAVEWESNGQPENNYKTTPPVLDSDGSFFLYSKLTVDKSRWQQGNVFSCSVMHEALHNHYTQKSLSLSPG

SEQ ID NO: 68 - protein, 449 aa, Artificial Sequence
  AM-9 full length IgG1 N297A heavy chain
EVQLVESGGGLVQPGGSLRLSCAASGFTFGGQQASWVRRAPGKGLEWVSAISGSGGSTYYADSVKGRFTISRDNSKNTLYLQMNSLRAEDTAVYYCAKGGDYGGNYFDYWGQGTLVTVSSASTKGPSVFPLAPSSKSTSGGTAALGCLVKDYFPEPVTVSWNSGALTSGVHTFPAVLQSSGLYSLSSVVTVPSSSLGTQTYICNVNHKPSNTKVDKRVEPKSCDKTHTCPPCPAPELLGGPSVFLFPPKPKDTLMISRTPEVTCVVVDVSHEDPEVKFNWYVDGVEVHNAKTKPREEQYASTYRVVSVLTVLHQDWLNGKEYKCKVSNKALPAPIEKTISKAKGQPREPQVYTLPPSREEMTKNQVSLTCLVKGFYPSDIAVEWESNGQPENNYKTTPPVLDSDGSFFLYSKLTVDKSRWQQGNVFSCSVMHEALHNHYTQKSLSLSPG

SEQ ID NO: 69 - protein, 214 aa, Artificial Sequence
  BADD466-3171 full length light chain sequence
EIVLTQSPATLSLSPGERATLSCRASQSVSSYLAWYQQKPGQAPRLLIYDASNRATGIPASFSGSGSGTDFTLTISRLEPEDFAVYYCQQYGSSPLTFGGGTKVEIKRTVAAPSVFIFPPSDEQLKSGTASVVCLLNNFYPREAKVQWKVDNALQSGNSQESVTEQDSKDSTYSLSSTLTLSKADYEKHKVYACEVTHQGLSSPVTKSFNRGEC

SEQ ID NO: 70 - protein, 329 aa, Artificial Sequence
  Human IgG1 G1m3 allotype (without C-terminal lysine)
ASTKGPSVFPLAPSSKSTSGGTAALGCLVKDYFPEPVTVSWNSGALTSGVHTFPAVLQSSGLYSLSSVVTVPSSSLGTQTYICNVNHKPSNTKVDKRVEPKSCDKTHTCPPCPAPELLGGPSVFLFPPKPKDTLMISRTPEVTCVVVDVSHEDPEVKFNWYVDGVEVHNAKTKPREEQYNSTYRVVSVLTVLHQDWLNGKEYKCKVSNKALPAPIEKTISKAKGQPREPQVYTLPPSREEMTKNQVSLTCLVKGFYPSDIAVEWESNGQPENNYKTTPPVLDSDGSFFLYSKLTVDKSRWQQGNVFSCSVMHEALHNHYTQKSLSLSPG

SEQ ID NO: 71 - protein, 330 aa, Artificial Sequence
  Human IgG1 G1m3 allotype
ASTKGPSVFPLAPSSKSTSGGTAALGCLVKDYFPEPVTVSWNSGALTSGVHTFPAVLQSSGLYSLSSVVTVPSSSLGTQTYICNVNHKPSNTKVDKRVEPKSCDKTHTCPPCPAPELLGGPSVFLFPPKPKDTLMISRTPEVTCVVVDVSHEDPEVKFNWYVDGVEVHNAKTKPREEQYNSTYRVVSVLTVLHQDWLNGKEYKCKVSNKALPAPIEKTISKAKGQPREPQVYTLPPSREEMTKNQVSLTCLVKGFYPSDIAVEWESNGQPENNYKTTPPVLDSDGSFFLYSKLTVDKSRWQQGNVFSCSVMHEALHNHYTQKSLSLSPGK

SEQ ID NO: 72 - protein, 329 aa, Artificial Sequence
  IgG1 N297A (without C-terminal lysine)
ASTKGPSVFPLAPSSKSTSGGTAALGCLVKDYFPEPVTVSWNSGALTSGVHTFPAVLQSSGLYSLSSVVTVPSSSLGTQTYICNVNHKPSNTKVDKRVEPKSCDKTHTCPPCPAPELLGGPSVFLFPPKPKDTLMISRTPEVTCVVVDVSHEDPEVKFNWYVDGVEVHNAKTKPREEQYASTYRVVSVLTVLHQDWLNGKEYKCKVSNKALPAPIEKTISKAKGQPREPQVYTLPPSREEMTKNQVSLTCLVKGFYPSDIAVEWESNGQPENNYKTTPPVLDSDGSFFLYSKLTVDKSRWQQGNVFSCSVMHEALHNHYTQKSLSLSPG

SEQ ID NO: 73 - protein, 330 aa, Artificial Sequence
  IgG1 N297A
ASTKGPSVFPLAPSSKSTSGGTAALGCLVKDYFPEPVTVSWNSGALTSGVHTFPAVLQSSGLYSLSSVVTVPSSSLGTQTYICNVNHKPSNTKVDKRVEPKSCDKTHTCPPCPAPELLGGPSVFLFPPKPKDTLMISRTPEVTCVVVDVSHEDPEVKFNWYVDGVEVHNAKTKPREEQYASTYRVVSVLTVLHQDWLNGKEYKCKVSNKALPAPIEKTISKAKGQPREPQVYTLPPSREEMTKNQVSLTCLVKGFYPSDIAVEWESNGQPENNYKTTPPVLDSDGSFFLYSKLTVDKSRWQQGNVFSCSVMHEALHNHYTQKSLSLSPGK

SEQ ID NO: 74 - protein, 326 aa, Artificial Sequence
  IgG4 S228P (without C-terminal lysine)
ASTKGPSVFPLAPCSRSTSESTAALGCLVKDYFPEPVTVSWNSGALTSGVHTFPAVLQSSGLYSLSSVVTVPSSSLGTKTYTCNVDHKPSNTKVDKRVESKYGPPCPPCPAPEFLGGPSVFLFPPKPKDTLMISRTPEVTCVVVDVSQEDPEVQFNWYVDGVEVHNAKTKPREEQFNSTYRVVSVLTVLHQDWLNGKEYKCKVSNKGLPSSIEKTISKAKGQPREPQVYTLPPSQEEMTKNQVSLTCLVKGFYPSDIAVEWESNGQPENNYKTTPPVLDSDGSFFLYSRLTVDKSRWQEGNVFSCSVMHEALHNHYTQKSLSLSLG

SEQ ID NO: 75 - protein, 327 aa, Artificial Sequence
  IgG4 S228P
ASTKGPSVFPLAPCSRSTSESTAALGCLVKDYFPEPVTVSWNSGALTSGVHTFPAVLQSSGLYSLSSVVTVPSSSLGTKTYTCNVDHKPSNTKVDKRVESKYGPPCPPCPAPEFLGGPSVFLFPPKPKDTLMISRTPEVTCVVVDVSQEDPEVQFNWYVDGVEVHNAKTKPREEQFNSTYRVVSVLTVLHQDWLNGKEYKCKVSNKGLPSSIEKTISKAKGQPREPQVYTLPPSQEEMTKNQVSLTCLVKGFYPSDIAVEWESNGQPENNYKTTPPVLDSDGSFFLYSRLTVDKSRWQEGNVFSCSVMHEALHNHYTQKSLSLSLGK

SEQ ID NO: 76 - protein, 107 aa, Artificial Sequence [sequence omitted]

SEQ ID NO: 77 - protein, 107 aa, Artificial Sequence
  Human kappa light chain constant region IGKC*01 Km3 allotype (with T109S mutation)
RSVAAPSVFIFPPSDEQLKSGTASVVCLLNNFYPREAKVQWKVDNALQSGNSQESVTEQDSKDSTYSLSSTLTLSKADYEKHKVYACEVTHQGLSSPVTKSFNRGEC

SEQ ID NO: 78 - protein, 301 aa, Homo sapiens
MFSHLPFDCVLLLLLLLLTRSSEVEYRAEVGQNAYLPCFYTPAAPGNLVPVCWGKGACPVFECGNVVLRTDERDVNYWTSRYWLNGDFRKGDVSLTIENVTLADSGIYCCRIQIPGIMNDEKFNLKLVIKPAKVTPAPTRQRDFTAAFPRMLTTRGHGPAETQTLGSLPDINLTQISTLANELRDSRLANDLRDSGATIRIGIYIGAGICAGLALALIFGALIFKWYSHSKEKIQNLSLISLANLPPSGLANAVAEGIRSEENIYTIEENVYEVEEPNEYYCYVSSRQQPSQPLGCRFAMP

SEQ ID NO: 79 - protein, 280 aa, Homo sapiens
SEVEYRAEVGQNAYLPCFYTPAAPGNLVPVCWGKGACPVFECGNVVLRTDERDVNYWTSRYWLNGDFRKGDVSLTIENVTLADSGIYCCRIQIPGIMNDEKFNLKLVIKPAKVTPAPTRQRDFTAAFPRMLTTRGHGPAETQTLGSLPDINLTQISTLANELRDSRLANDLRDSGATIRIGIYIGAGICAGLALALIFGALIFKWYSHSKEKIQNLSLISLANLPPSGLANAVAEGIRSEENIYTIEENVYEVEEPNEYYCYVSSRQQPSQPLGCRFAMP

SEQ ID NO: 80 - protein, 117 aa, Artificial Sequence
  pab1944w VH
QVQLVQSGAEVKKPGASVKVSCKASGYTFTSYWMHWVRQAPGQGLEWMGEINPSNGRTNYNEKFKTRVTITADTSTSTAYMELSSLRSEDTAVYYCARGYYLYFDYWGQGTLVTVSS

SEQ ID NO: 81 - protein, 107 aa, Artificial Sequence
  pab1944w VL
DIQMTQSPSSLSASVGDRVTITCHASQGIRINIGWYQQKPGKAPKLLIYHGTNLEDGVPSRFSGSGSGTDFTLTISSLQPEDFATYYCVQYGQFPWTFGQGTKLEIK

SEQ ID NO: 82 - protein, 118 aa, Artificial Sequence
  Hum11 VH
QVQLVQSGAEVKKPGSSVKVSCKASGYTFTSYNMHWVRQAPGQGLEWMGDIYPGNGDTSYNQKFKGRVTITADKSTSTVYMELSSLRSEDTAVYYCARVGGAFPMDYWGQGTTVTVSS

SEQ ID NO: 83 - protein, 111 aa, Artificial Sequence
  Hum11 VL
AIQLTQSPSSLSASVGDRVTITCRASESVEYYGTSLMQWYQQKPGKAPKLLIYAASNVESGVPSRFSGSGSGTDFTLTISSLQPEDFATYFCQQSRKDPSTFGGGTKVEIK

SEQ ID NO: 84 - protein, 98 aa, Homo sapiens
QVQLVESGGGLVQPGGSLRLSCAASGFTFSSYAMSWVRQAPGKGLEWVSAISGSGGSTYYADSVKGRFTISRDNSKNTLYLQMNSLRAEDTAVYYCAK

SEQ ID NO: 85 - protein, 95 aa, Homo sapiens
DIQMTQSPSSLSASVGDRVTITCRASQGISNYLAWYQQKPGKVPKLLIYAASTLQSGVPSRFSGSGSGTDFTLTISSLQPEDVATYYCQKYNSAP

SEQ ID NO: 86 - protein, 95 aa, Homo sapiens
EIVLTQSPATLSLSPGERATLSCRASQSVSSYLAWYQQKPGQAPRLLIYDASNRATGIPARFSGSGSGTDFTLTISSLEPEDFAVYYCQQRSNWP

SEQ ID NO: 87 - protein, 96 aa, Homo sapiens
EIVLTQSPGTLSLSPGERATLSCRASQSVSSSYLAWYQQKPGQAPRLLIYGASSRATGIPDRFSGSGSGTDFTLTISRLEPEDFAVYYCQQYGSSP

SEQ ID NO: 88 - protein, 96 aa, Homo sapiens
EIVLTQSPATLSLSPGERATLSCGASQSVSSSYLAWYQQKPGLAPRLLIYDASSRATGIPDRFSGSGSGTDFTLTISRLEPEDFAVYYCQQYGSSP

SEQ ID NO: 89 - protein, 446 aa, Artificial Sequence
  pab1944w (IgG1 N297A) full length heavy chain
QVQLVQSGAEVKKPGASVKVSCKASGYTFTSYWMHWVRQAPGQGLEWMGEINPSNGRTNYNEKFKTRVTITADTSTSTAYMELSSLRSEDTAVYYCARGYYLYFDYWGQGTLVTVSSASTKGPSVFPLAPSSKSTSGGTAALGCLVKDYFPEPVTVSWNSGALTSGVHTFPAVLQSSGLYSLSSVVTVPSSSLGTQTYICNVNHKPSNTKVDKRVEPKSCDKTHTCPPCPAPELLGGPSVFLFPPKPKDTLMISRTPEVTCVVVDVSHEDPEVKFNWYVDGVEVHNAKTKPREEQYASTYRVVSVLTVLHQDWLNGKEYKCKVSNKALPAPIEKTISKAKGQPREPQVYTLPPSREEMTKNQVSLTCLVKGFYPSDIAVEWESNGQPENNYKTTPPVLDSDGSFFLYSKLTVDKSRWQQGNVFSCSVMHEALHNHYTQKSLSLSPG

SEQ ID NO: 90 - protein, 214 aa, Artificial Sequence
  pab1944w (IgG1 N297A) full length light chain
DIQMTQSPSSLSASVGDRVTITCHASQGIRINIGWYQQKPGKAPKLLIYHGTNLEDGVPSRFSGSGSGTDFTLTISSLQPEDFATYYCVQYGQFPWTFGQGTKLEIKRTVAAPSVFIFPPSDEQLKSGTASVVCLLNNFYPREAKVQWKVDNALQSGNSQESVTEQDSKDSTYSLSSTLTLSKADYEKHKVYACEVTHQGLSSPVTKSFNRGEC

SEQ ID NO: 91 - protein, 444 aa, Artificial Sequence
  Hum11 (IgG4 S228P) full length heavy chain
QVQLVQSGAEVKKPGSSVKVSCKASGYTFTSYNMHWVRQAPGQGLEWMGDIYPGNGDTSYNQKFKGRVTITADKSTSTVYMELSSLRSEDTAVYYCARVGGAFPMDYWGQGTTVTVSSASTKGPSVFPLAPCSRSTSESTAALGCLVKDYFPEPVTVSWNSGALTSGVHTFPAVLQSSGLYSLSSVVTVPSSSLGTKTYTCNVDHKPSNTKVDKRVESKYGPPCPPCPAPEFLGGPSVFLFPPKPKDTLMISRTPEVTCVVVDVSQEDPEVQFNWYVDGVEVHNAKTKPREEQFNSTYRVVSVLTVLHQDWLNGKEYKCKVSNKGLPSSIEKTISKAKGQPREPQVYTLPPSQEEMTKNQVSLTCLVKGFYPSDIAVEWESNGQPENNYKTTPPVLDSDGSFFLYSRLTVDKSRWQEGNVFSCSVMHEALHNHYTQKSLSLSLG

SEQ ID NO: 92 - protein, 218 aa, Artificial Sequence
  Hum11 (IgG4 S228P) full length light chain
AIQLTQSPSSLSASVGDRVTITCRASESVEYYGTSLMQWYQQKPGKAPKLLIYAASNVESGVPSRFSGSGSGTDFTLTISSLQPEDFATYFCQQSRKDPSTFGGGTKVEIKRTVAAPSVFIFPPSDEQLKSGTASVVCLLNNFYPREAKVQWKVDNALQSGNSQESVTEQDSKDSTYSLSSTLTLSKADYEKHKVYACEVTHQGLSSPVTKSFNRGEC

SEQ ID NO: 93 - protein, 7 aa, Homo sapiens
PVFECGN

SEQ ID NO: 94 - protein, 18 aa, Homo sapiens
VCWGKGACPVFECGNVVL

SEQ ID NO: 95 - protein, 10 aa, Homo sapiens
RIQIPGIMND

SEQ ID NO: 96 - protein, 17 aa, Homo sapiens
RIQIPGIMNDEKFNLKL

SEQ ID NO: 97 - protein, 7 aa, Homo sapiens
EKFNLKL

SEQ ID NO: 98 - protein, 9 aa, Homo sapiens
PAAPGNLVP

SEQ ID NO: 99 - protein, 9 aa, Homo sapiens
GKGACPVFE

SEQ ID NO: 100 - protein, 8 aa, Homo sapiens
DFTAAFPR

SEQ ID NO: 101 - protein, 280 aa, Artificial Sequence
  Human TIM-3 F40A
SEVEYRAEVGQNAYLPCFYTPAAPGNLVPVCWGKGACPVAECGNVVLRTDERDVNYWTSRYWLNGDFRKGDVSLTIENVTLADSGIYCCRIQIPGIMNDEKFNLKLVIKPAKVTPAPTRQRDFTAAFPRMLTTRGHGPAETQTLGSLPDINLTQISTLANELRDSRLANDLRDSGATIRIGIYIGAGICAGLALALIFGALIFKWYSHSKEKIQNLSLISLANLPPSGLANAVAEGIRSEENIYTIEENVYEVEEPNEYYCYVSSRQQPSQPLGCRFAMP

SEQ ID NO: 102 - protein, 179 aa, Homo sapiens
SEVEYRAEVGQNAYLPCFYTPAAPGNLVPVCWGKGACPVFECGNVVLRTDERDVNYWTSRYWLNGDFRKGDVSLTIENVTLADSGIYCCRIQIPGIMNDEKFNLKLVIKPAKVTPAPTRQRDFTAAFPRMLTTRGHGPAETQTLGSLPDINLTQISTLANELRDSRLANDLRDSGATIR